European Patent Specification EP 3 891 180 B1, published July 24, 2024. Title: Humanised anti-IL17BR Antibody. Applicant: LIFEARC. Application PCT/EP2019/084083. The sequence listing filed with the application follows.

SEQUENCE LISTING (31 sequences)

SEQ ID NO: 1 - protein, 5 aa, Artificial Sequence
  VHCDR1
SYWMN

SEQ ID NO: 2 - protein, 17 aa, Artificial Sequence
  VHCDR2
  MISC_FEATURE (12)..(12): Xaa = N or A
  MISC_FEATURE (16)..(16): Xaa = K or Q
  MISC_FEATURE (17)..(17): Xaa = D or G
RIDPYDSEIQYXQKFXX

SEQ ID NO: 3 - protein, 9 aa, Artificial Sequence
  VHCDR3
SGGFDWFAY

SEQ ID NO: 4 - protein, 11 aa, Artificial Sequence
  VLCDR1
RASENINSNLA

SEQ ID NO: 5 - protein, 7 aa, Artificial Sequence
  VLCDR2
DVTNLAD

SEQ ID NO: 6 - protein, 9 aa, Artificial Sequence
  VLCDR3
QHFWGPPYT

SEQ ID NO: 7 - protein, 118 aa, Artificial Sequence
  VH sequence HA
EVQLVQSGAEVKKPGASVKVSCKTSGYTFISYWMNWVRQAPGQGLEWMGRIDPYDSEIQYNQKFKDRVTLTRDTSISTAYMELSRLRSDDTAVYYCATSGGFDWFAYWGQGTLVTVSS

SEQ ID NO: 8 - protein, 118 aa, Artificial Sequence
  VH sequence
  MISC_FEATURE (1)..(1): Xaa = Q or E
  MISC_FEATURE (24)..(24): Xaa = A or T
  MISC_FEATURE (61)..(61): Xaa = A or N
  MISC_FEATURE (65)..(65): Xaa = Q or K
  MISC_FEATURE (66)..(66): Xaa = G or D
  MISC_FEATURE (70)..(70): Xaa = M or L
XVQLVQSGAEVKKPGASVKVSCKXSGYTFISYWMNWVRQAPGQGLEWMGRIDPYDSEIQYXQKFXXRVTXTRDTSISTAYMELSRLRSDDTAVYYCARSGGFDWFAYWGQGTLVTVSS

SEQ ID NO: 9 - protein, 118 aa, Artificial Sequence
  VH sequence HJ
QVQLVQSGAEVKKPGASVKVSCKASGYTFISYWMNWVRQAPGQGLEWMGRIDPYDSEIQYNQKFKDRVTMTRDTSISTAYMELSRLRSDDTAVYYCARSGGFDWFAYWGQGTLVTVSS

SEQ ID NO: 10 - protein, 118 aa, Artificial Sequence
  VH sequence HH
EVQLVQSGAEVKKPGASVKVSCKTSGYTFISYWMNWVRQAPGQGLEWMGRIDPYDSEIQYNQKFKDRVTLTRDTSISTAYMELSRLRSDDTAVYYCARSGGFDWFAYWGQGTLVTVSS

SEQ ID NO: 11 - protein, 118 aa, Artificial Sequence
  VH sequence HI
EVQLVQSGAEVKKPGASVKVSCKTSGYTFISYWMNWVRQAPGQGLEWMGRIDPYDSEIQYAQKFQGRVTLTRDTSISTAYMELSRLRSDDTAVYYCARSGGFDWFAYWGQGTLVTVSS

SEQ ID NO: 12 - protein, 107 aa, Artificial Sequence
  VL sequence KA
DIQMTQSPSSLSASVGDRVTITCRASENINSNLAWYQQKPGKAPKLLLYDVTNLADGVPSRFSGSGSGTDYTLTISSLQPEDFATYYCQHFWRPPYTFGGGTKVEIK

SEQ ID NO: 13 - protein, 107 aa, Artificial Sequence
  VL sequence KE
DIQMTQSPSSLSASVGDRVTITCRASENINSNLAWYQQKPGKAPKLLLYDVTNLADGVPSRFSGSGSGTDYTLTISSLQPEDFATYYCQHFWGPPYTFGGGTKVEIK

SEQ ID NO: 14 - protein, 17 aa, Artificial Sequence
  VHCDR2 HJ and HH
RIDPYDSEIQYNQKFKD

SEQ ID NO: 15 - protein, 17 aa, Artificial Sequence
  VHCDR2 HI
RIDPYDSEIQYAQKFQG

SEQ ID NO: 16 - protein, 327 aa, Artificial Sequence
  Hinge stabilized IgG4 constant region
ASTKGPSVFPLAPCSRSTSESTAALGCLVKDYFPEPVTVSWNSGALTSGVHTFPAVLQSSGLYSLSSVVTVPSSSLGTKTYTCNVDHKPSNTKVDKRVESKYGPPCPPCPAPEFLGGPSVFLFPPKPKDTLMISRTPEVTCVVVDVSQEDPEVQFNWYVDGVEVHNAKTKPREEQFNSTYRVVSVLTVLHQDWLNGKEYKCKVSNKGLPSSIEKTISKAKGQPREPQVYTLPPSQEEMTKNQVSLTCLVKGFYPSDIAVEWESNGQPENNYKTTPPVLDSDGSFFLYSRLTVDKSRWQEGNVFSCSVMHEALHNHYTQKSLSLSLGK

SEQ ID NO: 17 - protein, 445 aa, Artificial Sequence
  D9HJ-IgG4* sequence
QVQLVQSGAEVKKPGASVKVSCKASGYTFISYWMNWVRQAPGQGLEWMGRIDPYDSEIQYNQKFKDRVTMTRDTSISTAYMELSRLRSDDTAVYYCARSGGFDWFAYWGQGTLVTVSSASTKGPSVFPLAPCSRSTSESTAALGCLVKDYFPEPVTVSWNSGALTSGVHTFPAVLQSSGLYSLSSVVTVPSSSLGTKTYTCNVDHKPSNTKVDKRVESKYGPPCPPCPAPEFLGGPSVFLFPPKPKDTLMISRTPEVTCVVVDVSQEDPEVQFNWYVDGVEVHNAKTKPREEQFNSTYRVVSVLTVLHQDWLNGKEYKCKVSNKGLPSSIEKTISKAKGQPREPQVYTLPPSQEEMTKNQVSLTCLVKGFYPSDIAVEWESNGQPENNYKTTPPVLDSDGSFFLYSRLTVDKSRWQEGNVFSCSVMHEALHNHYTQKSLSLSLGK

SEQ ID NO: 18 - protein, 118 aa, Artificial Sequence
  D9.2 VH
QVQLQQPGAELVRPGASVKLSCKTSGYTFISYWMNWVKQGPEQGLEWIGRIDPYDSEIQYNQKFKDKAILTVDKSSSAAYMQLISLTSEDSAVYYCARSGGFDWFAYWGQGTLVTVSA

SEQ ID NO: 19 - protein, 120 aa, Artificial Sequence
  EF178110
EVQLVESGAEVKKPGASVKVSCKTSGYTFIDYYIHWVRQAPGQGLEWMGWINPKSGGTNYARNLRDRVTLTRDTSINTAYMELSRLRSDDTALYYCATLYGDYRPIQDSWGQGTLVTVSS

SEQ ID NO: 20 - protein, 118 aa, Artificial Sequence
  D9 HB
EVQLVQSGAEVKKPGASVKVSCKTSGYTFISYWMNWVRQAPGQGLEWIGRIDPYDSEIQYNQKFKDKAILTVDTSISTAYMELSRLRSDDTAVYYCARSGGFDWFAYWGQGTLVTVSS

SEQ ID NO: 21 - protein, 118 aa, Artificial Sequence
  D9 HC
EVQLVQSGAEVKKPGASVKVSCKTSGYTFISYWMNWVRQAPGQGLEWIGRIDPYDSEIQYNQKFKDRVTLTRDTSISTAYMELSRLRSDDTAVYYCATSGGFDWFAYWGQGTLVTVSS

SEQ ID NO: 22 - protein, 118 aa, Artificial Sequence
  D9 HD
EVQLVQSGAEVKKPGASVKVSCKTSGYTFISYWMNWVRQAPGQGLEWMGRIDPYDSEIQYNQKFKDKVTLTRDTSISTAYMELSRLRSDDTAVYYCATSGGFDWFAYWGQGTLVTVSS

SEQ ID NO: 23 - protein, 118 aa, Artificial Sequence
  D9 HE
EVQLVQSGAEVKKPGASVKVSCKTSGYTFISYWMNWVRQAPGQGLEWMGRIDPYDSEIQYNQKFKDRATLTRDTSISTAYMELSRLRSDDTAVYYCATSGGFDWFAYWGQGTLVTVSS

SEQ ID NO: 24 - protein, 118 aa, Artificial Sequence
  D9 HF
EVQLVQSGAEVKKPGASVKVSCKTSGYTFISYWMNWVRQAPGQGLEWMGRIDPYDSEIQYNQKFKDRVILTRDTSISTAYMELSRLRSDDTAVYYCATSGGFDWFAYWGQGTLVTVSS

SEQ ID NO: 25 - protein, 118 aa, Artificial Sequence
  D9 HG
EVQLVQSGAEVKKPGASVKVSCKTSGYTFISYWMNWVRQAPGQGLEWMGRIDPYDSEIQYNQKFKDRVTLTVDTSISTAYMELSRLRSDDTAVYYCATSGGFDWFAYWGQGTLVTVSS

SEQ ID NO: 26 - protein, 107 aa, Artificial Sequence
  D9.2 VK
DIQMTQSPASLSVSVGETVTITCRASENINSNLAWYQQKKGKSPQLLVYDVTNLADGVPSRFSGSGSGTQYSLKINSLQSEDFGSYYCQHFWRPPYTFGGGTNLEIK

SEQ ID NO: 27 - protein, 107 aa, Artificial Sequence
  Y14869
DIQMTQSPSSLSASVGDRVTITCRASQGISNSLAWYQQKPGKAPKLLLYAASRLESGVPSRFSGSGSGTDYTLTISSLQPEDFATYYCQQYYSTPLTFGGGTKVEIK

SEQ ID NO: 28 - protein, 107 aa, Artificial Sequence
  D9_KB
DIQMTQSPSSLSASVGDRVTITCRASENINSNLAWYQQKPGKAPKLLVYDVTNLADGVPSRFSGSGSGTQYTLTISSLQPEDFATYYCQHFWRPPYTFGGGTKVEIK

SEQ ID NO: 29 - protein, 107 aa, Artificial Sequence
  D9_KC
DIQMTQSPSSLSASVGDRVTITCRASENINSNLAWYQQKPGKAPKLLVYDVTNLADGVPSRFSGSGSGTDYTLTISSLQPEDFATYYCQHFWRPPYTFGGGTKVEIK

SEQ ID NO: 30 - protein, 107 aa, Artificial Sequence
  D9_KD
DIQMTQSPSSLSASVGDRVTITCRASENINSNLAWYQQKPGKAPKLLLYDVTNLADGVPSRFSGSGSGTQYTLTISSLQPEDFATYYCQHFWRPPYTFGGGTKVEIK

SEQ ID NO: 31 - protein, 107 aa, Artificial Sequence
  KM
DIQMTQSPSSLSASVGDRVTITCRTSENIYSNLAWYQQKPGKAPKLLLYDATNLGDGVPSRFSGSGSGTDYTLTISSLQPEDFATYYCQHFWGPPYTFGGGTKVEIK